European Patent Application EP 4 245 774 A1, published September 20, 2023. Title: Fusion protein targeting both CD3 and CD137, preparation method therefor and use thereof. Applicant: Beijing Immunoah PharmaTech Co., Ltd. Application 21891172.5. The sequence listing filed with the application follows.

SEQUENCE LISTING (27 sequences)

SEQ ID NO: 1 - protein, 8 aa, Artificial Sequence
  SITE (1)..(1): Xaa may be any amino acid other than Cys, or is absent
XPPCPAPE

SEQ ID NO: 2 - protein, 8 aa, Artificial Sequence
  SITE (8)..(8): Xaa may be any amino acid other than Cys, or is absent
EPAPCPPX

SEQ ID NO: 3 - DNA, 363 bp, Artificial Sequence
gctagcaccaagggcccatccgtcttccccctggcaccctcctccaagagcacctctgggggcacagcggccctgggctgcctggtcaaggactacttccccgaaccggtgacggtgtcgtggaactcaggcgccctgaccagcggcgtgcacaccttcccggctgtcctacagtcctcaggactctactccctcagcagcgtggtgaccgtgccctccagcagcttgggcacccagacctacatctgcaacgtgaatcacaagcccagcaacaccaaggtggacaagaaagttgagcccaaatcttgtgacaaaactcacacaccaccgtgcccagcacctgaactcctggggggaccgtca

SEQ ID NO: 4 - DNA, 375 bp, Artificial Sequence
cgaactgtggctgcaccatctgtcttcatcttcccgccatctgatgagcagttgaaatctggaactgcctctgttgtgtgcctgctgaataacttctatcccagagaggccaaagtacagtggaaggtggataacgccctccaatcgggtaactcccaggagagtgtcacagagcaggacagcaaggacagcacctacagcctcagcagcaccctgacgctgagcaaagcagactacgagaaacacaaagtctacgcctgcgaagtcacccatcagggcctgagctcgcccgtcacaaagagcttcaacaggggagagtgtgacaaaactcacacaccaccgtgcccagcacctgaactcctggggggaccgtca

SEQ ID NO: 5 - DNA, 54 bp, Artificial Sequence
tcaccgggagggctgctcgaacctgcaccatgcccgccaacacacactaaagac

SEQ ID NO: 6 - DNA, 47 bp, Artificial Sequence
ggcacactggtcacagtttctagctcaccgggagggctgctcgaacc

SEQ ID NO: 7 - DNA, 47 bp, Artificial Sequence
ctgattatgatcaatgaattctcaagaggacactgtgaccagggtgc

SEQ ID NO: 8 - DNA, 46 bp, Artificial Sequence
ggaggcaccaagctgacagttttgtcaccgggagggctgctcgaac

SEQ ID NO: 9 - DNA, 49 bp, Artificial Sequence
ctgattatgatcaatgaattctcacttgatttccaccttggtgcctccg

SEQ ID NO: 10 - DNA, 44 bp, Artificial Sequence
tgtggctgagaggtgccagatgtcaagttcagctggttcagtct

SEQ ID NO: 11 - DNA, 47 bp, Artificial Sequence
gacggatgggcccttggtgctagcagaagagactgtgaccagggttc

SEQ ID NO: 12 - DNA, 47 bp, Artificial Sequence
gaaccctggtcacagtctcttctgctagcaccaagggcccatccgtc

SEQ ID NO: 13 - DNA, 47 bp, Artificial Sequence; identical to SEQ ID NO: 7

SEQ ID NO: 14 - DNA, 47 bp, Artificial Sequence
ctgtggctgagaggtgccagatgtgacgtggtcatgacacagagccc

SEQ ID NO: 15 - DNA, 48 bp, Artificial Sequence
gacagatggtgcagccacagttcgcttgatttccagcttggtgccctg

SEQ ID NO: 16 - DNA, 48 bp, Artificial Sequence
agggcaccaagctggaaatcaagcgaactgtggctgcaccatctgtct

SEQ ID NO: 17 - DNA, 49 bp, Artificial Sequence; identical to SEQ ID NO: 9

SEQ ID NO: 18 - DNA, 44 bp, Artificial Sequence
gtggctgagaggtgccagatgtgaggtccagctcgtcgagtccg

SEQ ID NO: 19 - DNA, 43 bp, Artificial Sequence
ggatgggcccttggtgctagcggcggaggagacggtgacgagg

SEQ ID NO: 20 - DNA, 43 bp, Artificial Sequence
ctcgtcaccgtctcctccgccgctagcaccaagggcccatccg

SEQ ID NO: 21 - DNA, 42 bp, Artificial Sequence
gtggctgagaggtgccagatgtgacatccagatgacccagtc

SEQ ID NO: 22 - DNA, 42 bp, Artificial Sequence
gatggtgcagccacagttcgcttgatctcgaccttggtgccc

SEQ ID NO: 23 - DNA, 44 bp, Artificial Sequence
gggcaccaaggtcgagatcaagcgaactgtggctgcaccatctg

SEQ ID NO: 24 - DNA, 42 bp, Artificial Sequence; identical to SEQ ID NO: 21

SEQ ID NO: 25 - DNA, 42 bp, Artificial Sequence
gctcttgggtgaccactgtctgacactctcccctgttgaagc

SEQ ID NO: 26 - DNA, 44 bp, Artificial Sequence; identical to SEQ ID NO: 18

SEQ ID NO: 27 - DNA, 43 bp, Artificial Sequence; identical to SEQ ID NO: 19